European Patent Specification EP 3 429 599 B1, published February 7, 2024. Title: NANOPARTICLE TO TARGET CANCER. Applicant: GEORGETOWN UNIVERSITY THE UNITED STATES OF AMERICA, AS REPRESENTED BY THE SECRETARY, DEPARTMENT OF HEALTH AND HUMAN SERVICES. The sequence listing filed with the application follows.

SEQUENCE LISTING (4 sequences)

SEQ ID NO: 1 - RNA, 19 nt, Artificial Sequence
  Synthetic oligonucleotide
gugcugaggaugagaacua

SEQ ID NO: 2 - RNA, 19 nt, Artificial Sequence
  Synthetic oligonucleotide
gaugcacccuuagguacag

SEQ ID NO: 3 - RNA, 19 nt, Artificial Sequence
  Synthetic oligonucleotide
agaagaagccuauggaugg

SEQ ID NO: 4 - DNA, 66 bp, Artificial Sequence
  Synthetic polynucleotide
catggtgcaggtgtggctgggattcatttgccggtgctggtgcgtccgcggccgctaatcctgttc